European Patent Specification EP 3 344 644 B1, published June 26, 2024. Title: CYCLIC DI-NUCLEOTIDE COMPOUNDS AS STING AGONISTS. Applicant: MERCK SHARP & DOHME CORP. The sequence listing filed with the application follows.

SEQUENCE LISTING (4 sequences)

SEQ ID NO: 1 - protein, 414 aa, Homo Sapien
MPHSSLHPSIPCPRGHGAQKAALVLLSACLVTLWGLGEPPEHTLRYLVLHLASLQLGLLLNGVCSLAEELHHIHSRYRGSYWRTVRACLGCPLRRGALLLLSIYFYYSLPNAVGPPFTWMLALLGLSQALNILLGLKGLAPAEISAVCEKGNFNVAHGLAWSYYIGYLRLILPELQARIRTYNQHYNNLLRGAVSQRLYILLPLDCGVPDNLSMADPNIRFLDKLPQQTADRAGIKDRVYSNSIYELLENGQRAGTCVLEYATPLQTLFAMSQYSQAGFSREDRLEQAKLFCQTLEDILADAPESQNNCRLIAYQEPADDSSFSLSQEVLRHLRQEEKEEVTVGSLKTSAVPSTSTMSQEPELLISGMEKPLPLRTDFSGGGLNDIFEAQKIEWHEGSLEVLFQGPHHHHHHHH

SEQ ID NO: 2 - DNA, 6482 bp, Homo Sapien
ggaacggctccgcccactattaatgaaattaaaaattccaattttaaaaaacgcagcaagagaaacatttgtatgaaagaatgcgtagaaggaaagaaaaatgtcgtcgacatgctgaacaacaagattaatatgcctccgtgtataaaaaaaatattgaacgatttgaaagaaaacaatgtaccgcgcggcggtatgtacaggaagaggtttatactaaactgttacattgcaaacgtggtttcgtgtgccaagtgtgaaaaccgatgtttaatcaaggctctgacgcatttctacaaccacgactccaagtgtgtgggtgaagtcatgcatcttttaatcaaatcccaagatgtgtataaaccaccaaactgccaaaaaatgaaaactgtcgacaagctctgtccgtttgctggcaactgcaagggtctcaatcctatttgtaattattgaataataaaacaattataaatgctaaatttgttttttattaacgatacaaaccaaacgcaacaagaacatttgtagtattatctataattgaaaacgcgtagttataatcgctgaggtaatatttaaaatcattttcaaatgattcacagttaatttgcgacaatataattttattttcacataaactagacgccttgtcgtcttcttcttcgtattccttctctttttcatttttctcttcataaaaattaacatagttattatcgtatccatatatgtatctatcgtatagagtaaattttttgttgtcataaatatatatgtcttttttaatggggtgtatagtaccgctgcgcatagtttttctgtaatttacaacagtgctattttctggtagttcttcggagtgtgttgctttaattattaaatttatataatcaatgaatttgggatcgtcggttttgtacaatatgttgccggcatagtacgcagcttcttctagttcaattacaccattttttagcagcaccggattaacataactttccaaaatgttgtacgaaccgttaaacaaaaacagttcacctcccttttctatactattgtctgcgagcagttgtttgttgttaaaaataacagccattgtaatgagacgcacaaactaatatcacaaactggaaatgtctatcaatatatagttgctgatcagatctgatcatggagataattaaaatgataaccatctcgcaaataaataagtattttactgttttcgtaacagttttgtaataaaaaaacctataaatataggatccatgccccactccagcctgcatccatccatcccgtgtcccaggggtcacggggcccagaaggcagccttggttctgctgagtgcctgcctggtgaccctttgggggctaggagagccaccagagcacactctccggtacctggtgctccacctagcctccctgcagctgggactgctgttaaacggggtctgcagcctggctgaggagctgcaccacatccactccaggtaccggggcagctactggaggactgtgcgggcctgcctgggctgccccctccgccgtggggccctgttgctgctgtccatctatttctactactccctcccaaatgcggtcggcccgcccttcacttggatgcttgccctcctgggcctctcgcaggcactgaacatcctcctgggcctcaagggcctggccccagctgagatctctgcagtgtgtgaaaaagggaatttcaacgtggcccatgggctggcatggtcatattacatcggatatctgcggctgatcctgccagagctccaggcccggattcgaacttacaatcagcattacaacaacctgctacggggtgcagtgagccagcggctgtatattctcctcccattggactgtggggtgcctgataacctgagtatggctgaccccaacattcgcttcctggataaactgccccagcagaccgctgaccgtgctggcatcaaggatcgggtttacagcaacagcatctatgagcttctggagaacgggcagcgggcgggcacctgtgtcctggagtacgccacccccttgcagactttgtttgccatgtcacaatacagtcaagctggctttagccgggaggataggcttgagcaggccaaactcttctgccagacacttgaggacatcctggcagatgcccctgagtctcagaacaactgccgcctcattgcctaccaggaacctgcagatgacagcagcttctcgctgtcccaggaggttctccggcacctgcggcaggaggaaaaggaagaggttactgtgggcagcttgaagacctcagcggtgcccagtacctccacgatgtcccaagagcctgagctcctcatcagtggaatggaaaagcccctccctctccgcacggatttctctggcggtggcctgaacgacatcttcgaagcccagaaaatcgaatggcatgaaggcagcctggaagtgctgttccagggcccacaccaccatcatcaccatcaccattaatgagcggccgcactcgagcaccaccaccaccaccactaacctaggtagctgagcgcatgcaagctgatccgggttattagtacatttattaagcgctagattctgtgcgttgttgatttacagacaattgttgtacgtattttaataattcattaaatttataatctttagggtggtatgttagagcgaaaatcaaatgattttcagcgtctttatatctgaatttaaatattaaatcctcaatagatttgtaaaataggtttcgattagtttcaaacaagggttgtttttccgaaccgatggctggactatctaatggattttcgctcaacgccacaaaacttgccaaatcttgtagcagcaatctagctttgtcgatattcgtttgtgttttgttttgtaataaaggttcgacgtcgttcaaaatattatgcgcttttgtatttctttcatcactgtcgttagtgtacaattgactcgacgtaaacacgttaaatagagcttggacatatttaacatcgggcgtgttagctttattaggccgattatcgtcgtcgtcccaaccctcgtcgttagaagttgcttccgaagacgattttgccatagccacacgacgcctattaattgtgtcggctaacacgtccgcgatcaaatttgtagttgagctttttggaattatttctgattgcgggcgtttttgggcgggtttcaatctaactgtgcccgattttaattcagacaacacgttagaaagcgatggtgcaggcggtggtaacatttcagacggcaaatctactaatggcggcggtggtggagctgatgataaatctaccatcggtggaggcgcaggcggggctggcggcggaggcggaggcggaggtggtggcggtgatgcagacggcggtttaggctcaaatgtctctttaggcaacacagtcggcacctcaactattgtactggtttcgggcgccgtttttggtttgaccggtctgagacgagtgcgatttttttcgtttctaatagcttccaacaattgttgtctgtcgtctaaaggtgcagcgggttgaggttccgtcggcattggtggagcgggcggcaattcagacatcgatggtggtggtggtggtggaggcgctggaatgttaggcacgggagaaggtggtggcggcggtgccgccggtataatttgttctggtttagtttgttcgcgcacgattgtgggcaccggcgcaggcgccgctggctgcacaacggaaggtcgtctgcttcgaggcagcgcttggggtggtggcaattcaatattataattggaatacaaatcgtaaaaatctgctataagcattgtaatttcgctatcgtttaccgtgccgatatttaacaaccgctcaatgtaagcaattgtattgtaaagagattgtctcaagctcggatcgatcccgcacgccgataacaagccttttcatttttactacagcattgtagtggcgagacacttcgctgtcgtcgaggtttaaacgcttcctcgctcactgactcgctgcgctcggtcgttcggctgcggcgagcggtatcagctcactcaaaggcggtaatacggttatccacagaatcaggggataacgcaggaaagaacatgtgagcaaaaggccagcaaaaggccaggaaccgtaaaaaggccgcgttgctggcgtttttccataggctccgcccccctgacgagcatcacaaaaatcgacgctcaagtcagaggtggcgaaacccgacaggactataaagataccaggcgtttccccctggaagctccctcgtgcgctctcctgttccgaccctgccgcttaccggatacctgtccgcctttctcccttcgggaagcgtggcgctttctcatagctcacgctgtaggtatctcagttcggtgtaggtcgttcgctccaagctgggctgtgtgcacgaaccccccgttcagcccgaccgctgcgccttatccggtaactatcgtcttgagtccaacccggtaagacacgacttatcgccactggcagcagccactggtaacaggattagcagagcgaggtatgtaggcggtgctacagagttcttgaagtggtggcctaactacggctacactagaaggacagtatttggtatctgcgctctgctgaagccagttaccttcggaaaaagagttggtagctcttgatccggcaaacaaaccaccgctggtagcggtggtttttttgtttgcaagcagcagattacgcgcagaaaaaaaggatctcaagaagatcctttgatcttttctacggggtctgacgctcagtggaacgaaaactcacgttaagggattttggtcatgagattatcaaaaaggatcttcacctagatccttttaaattaaaaatgaagttttaaatcaatctaaagtatatatgagtaaacttggtctgacagttaccaatgcttaatcagtgaggcacctatctcagcgatctgtctatttcgttcatccatagttgcctgactccccgtcgtgtagataactacgatacgggagggcttaccatctggccccagtgctgcaatgataccgcgagacccacgctcaccggctccagatttatcagcaataaaccagccagccggaagggccgagcgcagaagtggtcctgcaactttatccgcctccatccagtctattaattgttgccgggaagctagagtaagtagttcgccagttaatagtttgcgcaacgttgttgccattgctacaggcatcgtggtgtcacgctcgtcgtttggtatggcttcattcagctccggttcccaacgatcaaggcgagttacatgatcccccatgttgtgcaaaaaagcggttagctccttcggtcctccgatcgttgtcagaagtaagttggccgcagtgttatcactcatggttatggcagcactgcataattctcttactgtcatgccatccgtaagatgcttttctgtgactggtgagtactcaaccaagtcattctgagaatagtgtatgcggcgaccgagttgctcttgcccggcgtcaatacgggataataccgcgccacatagcagaactttaaaagtgctcatcattggaaaacgttcttcggggcgaaaactctcaaggatcttaccgctgttgagatccagttcgatgtaacccactcgtgcacccaactgatcttcagcatcttttactttcaccagcgtttctgggtgagcaaaaacaggaaggcaaaatgccgcaaaaaagggaataagggcgacacggaaatgttgaatactcatactcttcctttttcaatattattgaagcatttatcagggttattgtctcatgagcggatacatatttgaatgtatttagaaaaataaacaaataggggttccgcgcacatttccccgaaaagtgccacctgacgcgccctgtagcggcgcattaagcgcggcgggtgtggtggttacgcgcagcgtgaccgctacacttgccagcgccctagcgcccgctcctttcgctttcttcccttcctttctcgccacgttcgccggctttccccgtcaagctctaaatcgggggctccctttagggttccgatttagtgctttacggcacctcgaccccaaaaaacttgattagggtgatggttcacgtagtgggccatcgccctgatagacggtttttcgccctttgacgttggagtccacgttctttaatagtggactcttgttccaaactggaacaacactcaaccctatctcggtctattcttttgatttataagggattttgccgatttcggcctattggttaaaaaatgagctgatttaacaaaaatttaacgcgaattttaacaaaatattaacgtttacaatttcccattcgccattcaggctgcgcaactgttgggaagggcgatcggtgcgggcctcttcgctattacgcca

SEQ ID NO: 3 - protein, 414 aa, Homo Sapien
MPHSSLHPSIPCPRGHGAQKAALVLLSACLVTLWGLGEPPEHTLRYLVLHLASLQLGLLLNGVCSLAEELRHIHSRYRGSYWRTVRACLGCPLRRGALLLLSIYFYYSLPNAVGPPFTWMLALLGLSQALNILLGLKGLAPAEISAVCEKGNFNVAHGLAWSYYIGYLRLILPELQARIRTYNQHYNNLLRGAVSQRLYILLPLDCGVPDNLSMADPNIRFLDKLPQQTGDRAGIKDRVYSNSIYELLENGQRAGTCVLEYATPLQTLFAMSQYSQAGFSREDRLEQAKLFCRTLEDILADAPESQNNCRLIAYQEPADDSSFSLSQEVLRHLRQEEKEEVTVGSLKTSAVPSTSTMSQEPELLISGMEKPLPLRTDFSGGGLNDIFEAQKIEWHEGSLEVLFQGPHHHHHHHH

SEQ ID NO: 4 - DNA, 6482 bp, Homo Sapien
ggaacggctccgcccactattaatgaaattaaaaattccaattttaaaaaacgcagcaagagaaacatttgtatgaaagaatgcgtagaaggaaagaaaaatgtcgtcgacatgctgaacaacaagattaatatgcctccgtgtataaaaaaaatattgaacgatttgaaagaaaacaatgtaccgcgcggcggtatgtacaggaagaggtttatactaaactgttacattgcaaacgtggtttcgtgtgccaagtgtgaaaaccgatgtttaatcaaggctctgacgcatttctacaaccacgactccaagtgtgtgggtgaagtcatgcatcttttaatcaaatcccaagatgtgtataaaccaccaaactgccaaaaaatgaaaactgtcgacaagctctgtccgtttgctggcaactgcaagggtctcaatcctatttgtaattattgaataataaaacaattataaatgtcaaatttgttttttattaacgatacaaaccaaacgcaacaagaacatttgtagtattatctataattgaaaacgcgtagttataatcgctgaggtaatatttaaaatcattttcaaatgattcacagttaatttgcgacaatataattttattttcacataaactagacgccttgtcgtcttcttcttcgtattccttctctttttcatttttctcttcataaaaattaacatagttattatcgtatccatatatgtatctatcgtatagagtaaattttttgttgtcataaatatatatgtcttttttaatggggtgtatagtaccgctgcgcatagtttttctgtaatttacaacagtgctattttctggtagttcttcggagtgtgttgctttaattattaaatttatataatcaatgaatttgggatcgtcggttttgtacaatatgttgccggcatagtacgcagcttcttctagttcaattacaccattttttagcagcaccggattaacataactttccaaaatgttgtacgaaccgttaaacaaaaacagttcacctcccttttctatactattgtctgcgagcagttgtttgttgttaaaaataacagccattgtaatgagacgcacaaactaatatcacaaactggaaatgtctatcaatatatagttgctgatcagatctgatcatggagataattaaaatgataaccatctcgcaaataaataagtattttactgttttcgtaacagttttgtaataaaaaaacctataaatataggatccatgccccactccagcctgcatccatccatcccgtgtcccaggggtcacggggcccagaaggcagccttggttctgctgagtgcctgcctggtgaccctttgggggctaggagagccaccagagcacactctccggtacctggtgctccacctagcctccctgcagctgggactgctgttaaacggggtctgcagcctggctgaggagctgcgccacatccactccaggtaccggggcagctactggaggactgtgcgggcctgcctgggctgccccctccgccgtggggccctgttgctgctgtccatctatttctactactccctcccaaatgcggtcggcccgcccttcacttggatgcttgccctcctgggcctctcgcaggcactgaacatcctcctgggcctcaagggcctggccccagctgagatctctgcagtgtgtgaaaaagggaatttcaacgtggcccatgggctggcatggtcatattacatcggatatctgcggctgatcctgccagagctccaggcccggattcgaacttacaatcagcattacaacaacctgctacggggtgcagtgagccagcggctgtatattctcctcccattggactgtggggtgcctgataacctgagtatggctgaccccaacattcgcttcctggataaactgccccagcagaccggtgaccgtgctggcatcaaggatcgggtttacagcaacagcatctatgagcttctggagaacgggcagcgggcgggcacctgtgtcctggagtacgccacccccttgcagactttgtttgccatgtcacaatacagtcaagctggctttagccgggaggataggcttgagcaggccaaactcttctgccggacacttgaggacatcctggcagatgcccctgagtctcagaacaactgccgcctcattgcctaccaggaacctgcagatgacagcagcttctcgctgtcccaggaggttctccggcacctgcggcaggaggaaaaggaagaggttactgtgggcagcttgaagacctcagcggtgcccagtacctccacgatgtcccaagagcctgagctcctcatcagtggaatggaaaagcccctccctctccgcacggatttctctggcggtggcctgaacgacatcttcgaagcccagaaaatcgaatggcatgaaggcagcctggaagtgctgttccagggcccacaccaccatcatcaccatcaccattaatgagcggccgcactcgagcaccaccaccaccaccactaacctaggtagctgagcgcatgcaagctgatccgggttattagtacatttattaagcgctagattctgtgcgttgttgatttacagacaattgttgtacgtattttaataattcattaaatttataatctttagggtggtatgttagagcgaaaatcaaatgattttcagcgtctttatatctgaatttaaatattaaatcctcaatagatttgtaaaataggtttcgattagtttcaaacaagggttgtttttccgaaccgatggctggactatctaatggattttcgctcaacgccacaaaacttgccaaatcttgtagcagcaatctagctttgtcgatattcgtttgtgttttgttttgtaataaaggttcgacgtcgttcaaaatattatgcgcttttgtatttctttcatcactgtcgttagtgtacaattgactcgacgtaaacacgttaaatagagcttggacatatttaacatcgggcgtgttagctttattaggccgattatcgtcgtcgtcccaaccctcgtcgttagaagttgcttccgaagacgattttgccatagccacacgacgcctattaattgtgtcggctaacacgtccgcgatcaaatttgtagttgagctttttggaattatttctgattgcgggcgtttttgggcgggtttcaatctaactgtgcccgattttaattcagacaacacgttagaaagcgatggtgcaggcggtggtaacatttcagacggcaaatctactaatggcggcggtggtggagctgatgataaatctaccatcggtggaggcgcaggcggggctggcggcggaggcggaggcggaggtggtggcggtgatgcagacggcggtttaggctcaaatgtctctttaggcaacacagtcggcacctcaactattgtactggtttcgggcgccgtttttggtttgaccggtctgagacgagtgcgatttttttcgtttctaatagcttccaacaattgttgtctgtcgtctaaaggtgcagcgggttgaggttccgtcggcattggtggagcgggcggcaattcagacatcgatggtggtggtggtggtggaggcgctggaatgttaggcacgggagaaggtggtggcggcggtgccgccggtataatttgttctggtttagtttgttcgcgcacgattgtgggcaccggcgcaggcgccgctggctgcacaacggaaggtcgtctgcttcgaggcagcgcttggggtggtggcaattcaatattataattggaatacaaatcgtaaaaatctgctataagcattgtaatttcgctatcgtttaccgtgccgatatttaacaaccgctcaatgtaagcaattgtattgtaaagagattgtctcaagctcggatcgatcccgcacgccgataacaagccttttcatttttactacagcattgtagtggcgagacacttcgctgtcgtcgaggtttaaacgcttcctcgctcactgactcgctgcgctcggtcgttcggctgcggcgagcggtatcagctcactcaaaggcggtaatacggttatccacagaatcaggggataacgcaggaaagaacatgtgagcaaaaggccagcaaaaggccaggaaccgtaaaaaggccgcgttgctggcgtttttccataggctccgcccccctgacgagcatcacaaaaatcgacgctcaagtcagaggtggcgaaacccgacaggactataaagataccaggcgtttccccctggaagctccctcgtgcgctctcctgttccgaccctgccgcttaccggatacctgtccgcctttctcccttcgggaagcgtggcgctttctcatagctcacgctgtaggtatctcagttcggtgtaggtcgttcgctccaagctgggctgtgtgcacgaaccccccgttcagcccgaccgctgcgccttatccggtaactatcgtcttgagtccaacccggtaagacacgacttatcgccactggcagcagccactggtaacaggattagcagagcgaggtatgtaggcggtgctacagagttcttgaagtggtggcctaactacggctacactagaaggacagtatttggtatctgcgctctgctgaagccagttaccttcggaaaaagagttggtagctcttgatccggcaaacaaaccaccgctggtagcggtggtttttttgtttgcaagcagcagattacgcgcagaaaaaaaggatctcaagaagatcctttgatcttttctacggggtctgacgctcagtggaacgaaaactcacgttaagggattttggtcatgagattatcaaaaaggatcttcacctagatccttttaaattaaaaatgaagttttaaatcaatctaaagtatatatgagtaaacttggtctgacagttaccaatgcttaatcagtgaggcacctatctcagcgatctgtctatttcgttcatccatagttgcctgactccccgtcgtgtagataactacgatacgggagggcttaccatctggccccagtgctgcaatgataccgcgagacccacgctcaccggctccagatttatcagcaataaaccagccagccggaagggccgagcgcagaagtggtcctgcaactttatccgcctccatccagtctattaattgttgccgggaagctagagtaagtagttcgccagttaatagtttgcgcaacgttgttgccattgctacaggcatcgtggtgtcacgctcgtcgtttggtatggcttcattcagctccggttcccaacgatcaaggcgagttacatgatcccccatgttgtgcaaaaaagcggttagctccttcggtcctccgatcgttgtcagaagtaagttggccgcagtgttatcactcatggttatggcagcactgcataattctcttactgtcatgccatccgtaagatgcttttctgtgactggtgagtactcaaccaagtcattctgagaatagtgtatgcggcgaccgagttgctcttgcccggcgtcaatacgggataataccgcgccacatagcagaactttaaaagtgctcatcattggaaaacgttcttcggggcgaaaactctcaaggatcttaccgctgttgagatccagttcgatgtaacccactcgtgcacccaactgatcttcagcatcttttactttcaccagcgtttctgggtgagcaaaaacaggaaggcaaaatgccgcaaaaaagggaataagggcgacacggaaatgttgaatactcatactcttcctttttcaatattattgaagcatttatcagggttattgtctcatgagcggatacatatttgaatgtatttagaaaaataaacaaataggggttccgcgcacatttccccgaaaagtgccacctgacgcgccctgtagcggcgcattaagcgcggcgggtgtggtggttacgcgcagcgtgaccgctacacttgccagcgccctagcgcccgctcctttcgctttcttcccttcctttctcgccacgttcgccggctttccccgtcaagctctaaatcgggggctccctttagggttccgatttagtgctttacggcacctcgaccccaaaaaacttgattagggtgatggttcacgtagtgggccatcgccctgatagacggtttttcgccctttgacgttggagtccacgttctttaatagtggactcttgttccaaactggaacaacactcaaccctatctcggtctattcttttgatttataagggattttgccgatttcggcctattggttaaaaaatgagctgatttaacaaaaatttaacgcgaattttaacaaaatattaacgtttacaatttcccattcgccattcaggctgcgcaactgttgggaagggcgatcggtgcgggcctcttcgctattacgcca